European Patent Application EP 4 803 159 A2, published September 9, 2026. Title: CONJUGATE OF SALICYLIC ACID AND PEPTIDE. Applicant: CAREGEN CO., LTD. Application EP, filed February 16, 2017. The sequence listing filed with the application follows.

SEQUENCE LISTING (18 sequences)

SEQ ID NO: 1 - protein, 10 aa, synthetic construct
  REGION 1..10: note = Peptide 1
YKSKKGGWTH

SEQ ID NO: 2 - protein, 12 aa, synthetic construct
  REGION 1..12: note = Peptide 2
YISKKHAGKNWF

SEQ ID NO: 3 - protein, 8 aa, synthetic construct
  REGION 1..8: note = Peptide 3
KLKKTETQ

SEQ ID NO: 4 - protein, 12 aa, synthetic construct
  REGION 1..12: note = Peptide 4
ELIEHGGGRPAD

SEQ ID NO: 5 - DNA, 20 bp, synthetic construct
  misc_feature 1..20: note = forward primer for collagen
  source 1..20: mol_type = other DNA
caccctcaagagcctgagtc

SEQ ID NO: 6 - DNA, 20 bp, synthetic construct
  misc_feature 1..20: note = reverse primer for collagen
  source 1..20: mol_type = other DNA
agacggctgagtagggaaca

SEQ ID NO: 7 - DNA, 20 bp, synthetic construct
  misc_feature 1..20: note = forward primer for elastin
  source 1..20: mol_type = other DNA
ggacccctgactcgcgacct

SEQ ID NO: 8 - DNA, 20 bp, synthetic construct
  misc_feature 1..20: note = reverse primer for elastin
  source 1..20: mol_type = other DNA
ggggaggtgggactgcccaa

SEQ ID NO: 9 - DNA, 20 bp, synthetic construct
  misc_feature 1..20: note = forward primer for fibronectin
  source 1..20: mol_type = other DNA
ccaggaaccgagtacaccat

SEQ ID NO: 10 - DNA, 20 bp, synthetic construct
  misc_feature 1..20: note = reverse primer for fibronectin
  source 1..20: mol_type = other DNA
atacccaggttgggtgatga

SEQ ID NO: 11 - DNA, 21 bp, synthetic construct
  misc_feature 1..21: note = forward primer for TNF-alpha
  source 1..21: mol_type = other DNA
cgtcagccgattrtgctatct

SEQ ID NO: 12 - DNA, 20 bp, synthetic construct
  misc_feature 1..20: note = reverse primer for TNF-alpha
  source 1..20: mol_type = other DNA
cggactccgcaaagtctaag

SEQ ID NO: 13 - DNA, 20 bp, synthetic construct
  misc_feature 1..20: note = forward primer for IL-6
  source 1..20: mol_type = other DNA
aaagaggcactgccagaaaa

SEQ ID NO: 14 - DNA, 20 bp, synthetic construct
  misc_feature 1..20: note = reverse primer for IL-6
  source 1..20: mol_type = other DNA
atctgaggtgcccatgctac

SEQ ID NO: 15 - DNA, 20 bp, synthetic construct
  misc_feature 1..20: note = forward primer for IL-1b
  source 1..20: mol_type = other DNA
ttcgacacatgggataacga

SEQ ID NO: 16 - DNA, 20 bp, synthetic construct
  misc_feature 1..20: note = reverse primer for IL-1b
  source 1..20: mol_type = other DNA
tctttcaacacgcaggacag

SEQ ID NO: 17 - DNA, 21 bp, synthetic construct
  misc_feature 1..21: note = forward primer for COX-2
  source 1..21: mol_type = other DNA
atcattcaccaggcaaattgc

SEQ ID NO: 18 - DNA, 21 bp, synthetic construct
  misc_feature 1..21: note = reverse primer for COX-2
  source 1..21: mol_type = other DNA
ggcttcagcataaagcgtttg